European Patent Application EP 4 631 511 A1, published October 15, 2025. Title: Probiotic Strains and Uses thereof. Applicant: SICHUAN ANAEROBIC BIOTECHNOLOGY CO., LTD. Application CN. The sequence listing filed with the application follows.

SEQUENCE LISTING (8 sequences)

SEQ ID NO: 1 - DNA, 19 bp, synthetic construct
  source 1..19: mol_type = other DNA
agttgacggaccccaaaag

SEQ ID NO: 2 - DNA, 20 bp, synthetic construct
  source 1..20: mol_type = other DNA
agctggatgctctcatcagg

SEQ ID NO: 3 - DNA, 19 bp, synthetic construct
  source 1..19: mol_type = other DNA
ctgtagcccacgtcgtagc

SEQ ID NO: 4 - DNA, 18 bp, synthetic construct
  source 1..18: mol_type = other DNA
ttgagatccatgccgttg

SEQ ID NO: 5 - DNA, 23 bp, synthetic construct
  source 1..23: mol_type = other DNA
ggaacatcagcggtggacacttc

SEQ ID NO: 6 - DNA, 22 bp, synthetic construct
  source 1..22: mol_type = other DNA
gggaattagcatggtcttgagg

SEQ ID NO: 7 - DNA, 20 bp, synthetic construct
  source 1..20: mol_type = other DNA
ctcaacacgggaaacctcac

SEQ ID NO: 8 - DNA, 20 bp, synthetic construct
  source 1..20: mol_type = other DNA
cgctccaccaactaagaacg